European Patent Specification EP 3 917 551 B1, published April 22, 2026. Title: LACTOCOCCUS LACTIS STRAINS FOR THE PREVENTION AND/OR THE TREATMENT OF VISCERAL PAIN. Applicant: INSTITUT NATIONAL DE RECHERCHE POUR L'AGRICULTURE, L'ALIMENTATION ET L'ENVIRONNEMENT INSTITUT NATIONAL DES SCIENCES APPLIQUEES DE TOULOUSE CENTRE NATIONAL DE LA RECHERCHE SCIENTIFIQUE ECOLE D'INGENIEURS DE PURPAN ECOLE NATIONALE VETERINAIRE DE TOULOUSE UNIVERSITE TOULOUSE III - PAUL SABATIER COGAIGN-BOUSQUET, Muriel EUTAMENE, Hélène MERCIER-BONIN, Muriel THEODOROU, Vassilia LAROUTE, Valérie DAVERAN-MINGOT, Marie-Line. The sequence listing filed with the application follows.

SEQUENCE LISTING (13 sequences)

SEQ ID NO: 1 - DNA, 33 bp, Lactococcus lactis
ggaattcgatttagatgccataggaggattttc

SEQ ID NO: 2 - DNA, 33 bp, Lactococcus lactis
gatgaatatcgtacatcctccaattttttaatg

SEQ ID NO: 3 - DNA, 37 bp, Lactococcus lactis
aagcttgataaaacaagaaaatattcatgaaattcag

SEQ ID NO: 4 - DNA, 39 bp, Lactococcus lactis
ggaggatgtacgatattcatcttaagaaaaatcaaaagc

SEQ ID NO: 5 - DNA, 26 bp, Lactococcus lactis
catctaaatcgaattcctgcagcccg

SEQ ID NO: 6 - DNA, 30 bp, Lactococcus lactis
tcttgttttatcaagcttatcgataccgtc

SEQ ID NO: 7 - DNA, 27 bp, Lactococcus lactis
ttggattagctgcggcatattttatcg

SEQ ID NO: 8 - DNA, 27 bp, Lactococcus lactis
ccttgttgaccataatgcaaagcaggt

SEQ ID NO: 9 - DNA, 30 bp, Lactococcus lactis
aaaatatagaaggagactattgcaaatagc

SEQ ID NO: 10 - DNA, 30 bp, Lactococcus lactis
aaaaattaatggccatcgttggtagttctc

SEQ ID NO: 11 - DNA, 29 bp, Lactococcus lactis
tctgtgcagcagaaatggcgacggttgaa

SEQ ID NO: 12 - DNA, 30 bp, Lactococcus lactis
tccccataaatttttctttttcactcgcat

SEQ ID NO: 13 - DNA, 30 bp, Lactococcus lactis
cggttattcctcaaaaagacttatcattaa